European Patent Application EP 4 190 349 A2, published June 7, 2023. Title: PRODUCTION OF EXOSOMES AND USES THEREOF. Applicant: China Medical University. Application EP. The sequence listing filed with the application follows.

SEQUENCE LISTING (2 sequences)

SEQ ID NO: 1 - DNA, 405 bp, synthetic construct
  source 1..405: mol_type = other DNA
agcgctggtcacgtgcagctggtggaaagcggcggcggcagcgtgcaagccggcggcagcctgaagctgagctgcgtgacaagcgcctacaccttctccgctagcggcaactgcatgggctggctgagacaagcccccggcaagggcagagagggcatcgccgccacctacacaagaagcgccaagacctactacgccgacagcgtgaagggcagattcaccatcagccaagacaacgccaagaacaccgtgtacctgcagatgaacggcctgaagcccgaggacaccgccacctactactgcgccgtggctagatgcgccggcagacccgacagaagcaccctgacaagcttcgcctggtggggccaaggcacccaagtgaccgtgagcagcctggagaccggt

SEQ ID NO: 2 - protein, 135 aa, synthetic construct
SAGHVQLVESGGGSVQAGGSLKLSCVTSAYTFSASGNCMGWLRQAPGKGREGIAATYTRSAKTYYADSVKGRFTISQDNAKNTVYLQMNGLKPEDTATYYCAVARCAGRPDRSTLTSFAWWGQGTQVTVSSLETG